European Patent Specification EP 2 597 152 B1, published November 1, 2023. Title: A genetically engineered bacterial strain WSJ-IA I producing high content          and high yield of isovaleryl spiramycin. Applicant: Shen Yang Tonglian Group Co.,Ltd. The sequence listing filed with the application follows.

SEQUENCE LISTING (6 sequences)

SEQ ID NO: 1 - DNA, 1393 bp, Streptomyces spiramyceticus
  16S rDNA (20)..(1413)
ccttcgacagctccctcccacaaggggttgggccaccggcttcgggtgttaccgactttcgtgacgtgacgggcggtgtgtacaaggcccgggaacgtattcaccgcagcaatgctgatctgcgattactagcaactccgacttcatggggtcgagttgcagaccccaatccgaactgagaccggctttttgagattcgctccgcctcgcggcatcgcagctcattgtacggccattgtagcacgtgtgcagcccaagacataaggggcatgatgacttgacgtcgtccccaccttcctccgagttgaccccggcggtctcctgtgagtccccatcaccccgaagggcatgctggcaacacaggacaagggttgcgctcgttgcgggacttaacccaacatctcacgacacgagctgacgacagccatgcaccacctgtataccgaccacaagggggcacctatctctaggtgtttccggtatatgtcaagccttggtaaggttcttcgcgttgcgtcgaattaagccacatgctccgctgcttgtgcgggcccccgtcaattcctttgagttttagccttgcggccgtactccccaggcggggaacttaatgcgttagctgcggcaccgacgacgtggaatgtcgccaacacctagttcccaacgtttacggcgtggactaccagggtatctaatcctgttcgctccccacgctttcgctcctcagcgtcagtaatggcccagagatccgccttcgccaccggtgttcctcctgatatctgcgcatttcaccgctacaccaggaattccgatctcccctaccacactctagcctgcccgtatcgaatgcagacccggggttaagccccgggctttcacatccgacgcgacaagccgcctacgagctctttacgcccaataattccggacaacgcttgcgccctacgtattaccgcggctgctggcacgtagttagccggcgcttcttctgcaggtaccgtcactttcgcttcttccctgctgaaagaggtttacaacccgaaggccgtcatccctcacgcggcgtcgctgcatcaggctttcgcccattgtgcaatattccccactgctgcctcccgtaggagtctgggccgtgtctcagtcccagtgtggccggtcgccctctcaggccggctacccgtcgtcgccttggtaggccattaccccaccaacaagctgataggccgcgggctcatccttcaccgccggagcttttaacccccacccatgcaggcaggagtgttatccggtattagaccccgtttccagggcttgtcccagagtgaagggcagattgcccacgtgttactcacccgttcgccactaatccaccccgaagggcttcatcgttcga

SEQ ID NO: 2 - DNA, 680 bp, Streptomyces spiramyceticus
  atpD (553)..(1232)
agcttgtcctcttcgcccagctcgtcgataccgaggatcgcgatgatgtcctggaggtccttgtacttctgcaggattcccttgacgcggctggccgcgtcgtagtggtcctgcgtgatgtagcgggggtccaggatgcgggacgtcgagtccagcgggtcgaccgccgggtagatgcccttctccgagatcgggcgcgacagaacggtcgtcgcgtccaggtgggcgaaggtggtcgccggcgccgggtcggtcaggtcgtccgcggggacgtagatcgcctgcatcgaggtgatcgagtgaccacgcgtcgaggtgatgcgctcctggagcacacccatctcgtcggccagggtcggctggtaacccactgcggacggcatacggccgagcagcgtggagacctcggaaccggcctgggtgaagcggaagatgttgtcgatgaagagcagcacgtcctgcttctgaacatcgcggaagtactccgccatggtcagggcggacagggcgacgcgcagacgcgtgcccggcggctcgtccatctggccgaagaccagcgcggtcttgtccagaacacccgattcggtcatctcgtcgatgaggtcgttgccctcacgggtgcgctcgccgacaccggcgaacaccgacacaccctcgtgcagcttcgccacacgcatgat

SEQ ID NO: 3 - DNA, 1177 bp, Streptomyces spiramyceticus
  gryB (20)..(1196)
ccggcggtctgcacggcgtcggcgtctccgtggtgaacgcgctgtcgtcgaaggtcgctgtcgaggtcaagcgcgacggttaccgctggacgcaggactacaagctcggtgtgccgacggcgccgctggcccgtaacgaggccacggaggagtccggtacctctgtcaccttctgggccgacccggacgtcttcgagacgaccgactactccttcgagacgctgtcgcggcgtttccaggagatggcgttcctcaacaagggcctgacgctcaagctgacggacgagcgggagtccgcgaaggccgtggcgggggcggacacggcggacggtacggaggacgaccaggtccgtacggtcacgtaccactacgaaggcggcatcgtcgacttcgtgaagtacctgaactcgcgcaagggtgagctgattcacccgaccgtcatcgacgtcgaggccgaggacaaggagcgcatgctctcggtcgagatcgcgatgcagtggaactcgcagtacaccgagggtgtctactccttcgcgaacacgatccacacgcacgagggcggcacgcacgaagagggcttccgtgcggcgatgacaggtctggtcaaccggtacgcgcgcgagaagaagttcctgcgtgagaaggacgacaacctcgccggtgaggacatccgtgagggtctgacggcgatcatctcgatcaagctgggcgagccgcagttcgagggtcagacgaagaccaagctgggcaacacggaggcgaagaccttcgtgcagaaggtcgtgcacgagcacctcaacgactggttcgaccgcaatccgaacgaggccgcggacatcatccgcaagtcgatccaggcggccacggcgcgcgtcgcggcccgcaaggcgcgcgacctgacccgtcgcaagggcctgctggagtcggcctcgctgccgggcaagctgtccgactgccagtcgaacgacccgacgaagtgcgagatcttcatcgtcgagggtgactccgccggtggctcggcgaagtccggtcgtaacccgatgtaccaggccatcctgccgatccgaggcaagatcctgaacgtcgagaaggcgcggatcgacaagatcctccagaacaccgaggtccaggcgctgatctcggcgttcggcacgggtgtgcacgaggacttcgacat

SEQ ID NO: 4 - DNA, 870 bp, Streptomyces spiramyceticus
  gryB (1276)..(2145)
gtcgtcgcctccatcaaggagttcttcggcaccacccagctgtcgcagttcatggaccagaacaacccgctgtcgggtctcacccacaagcgccgtctgtcggcgcttggcccgggtggtctctcccgtgagcgggccggcttcgaggtccgtgacgtgcacccgtctcactacggccgcatgtgcccgattgagacccctgaaggcccgaacatcggtctgatcggttcgctcgcctcgtacggccgcgtcaacgcgttcggcttcgtcgagacgccgtaccgcaaggtcgtcgacggtgtcgtcaccgacgacgtcgactacctgacggccgacgaagaggaccgcttcgtcatcgcgcaggccaacgcgacgctctccgaggacatgcgcttcgaggagtcccgcgtcctggtccgccgtcgtggcggcgagatcgactacatcccgggcgacgacgtcgactacatggacgtctcgccgcgccagatggtgtcggtcgcgaccgcgatgatcccgttcctcgagcacgacgacgcaaaccgcgcgctcatgggcgcgaacatgatgcgtcaggccgtgccgctgatcacgtccgaggcgccgctcgtcggcaccggcatggaataccgctgtgcggtcgacgccggtgacgtcatcaaggcggagaaggagggcgtggtccaggaggtttccgcggactacgtcaccgtcgccaacgacgacggtacgtacaccacgtaccgcatcgccaagttctcccgctccaaccagggcacctcggtcaaccagaaggttgtcgtcgacgagggtgcccgggtcgtcgagggccaggtcctcgccgacgggcccgccacccagcagggtgag

SEQ ID NO: 5 - DNA, 701 bp, Streptomyces spiramyceticus
  gryB (167)..(867)
accggccgacgaccccatcgaggtcatctccaccgggtcgaccgctctggacatcgcgctcggcgtcggcggactgccgcgcggtcgtgtggtggaggtgtacggaccggaatcctccggtaagacgacactgacgctgcacgccgtggccaacgcgcagaaggccggtggcaccgtcgccttcgtggatgccgagcacgcgctcgaccccgaatacgccaaggcactcggcgtcgacacggacaatctgatcctctcccagccggacaccggcgagcaggccctcgagatcgtggacatgctggtccgctcgggcgccatcgacctcatcgtcattgactccgtcgccgccctggtgccgcgcgcggagattgagggtgagatgggcgactcgcacgtcggcctccaggcccggctgatgagccaggcgctgcgcaagatcactggcgcgctgcaccagtcccagaccacagcgatcttcatcaaccagctccgcgagaagatcggtgtgatgttcggctccccggagaccacgacaggtggccgggcgctgaagttctacgcctccgtgcggctcgacatccgccgtatcgagaccctcaaggacggcacggacgcggtcggcaaccgcacccgcgtcaaggtcgtcaaaaacaaggtcgcgccgccgttcaagcaggccgagttcgacatcctctacg

SEQ ID NO: 6 - DNA, 611 bp, Streptomyces spiramyceticus
  trpB (1)..(611)
gctcaccaagcgcatgggcaagacgcgcgtgatcgcggagaccggcgccggccagcacggcgtcgccaccgccaccgcgtgcgccctcttcggcctcgaatgcaccatctacatgggcgagatcgacaccgagcgccaggcgctcaacgtcgcccgcatgcggatgctcggtgccgaggtcgtcgccgtgaagtccggcagccgcaccctgaaggacgccatcaacgaggcgttccgcgactgggtcgccaatgtcgaccgtacgcactacctcttcggcacggtcgccggcccgcaccccttccccgccatggtccgcgacttccaccgggtcatcggtgtcgaggcacgccgccagatcctggagcgcacgggacggctgcccgacgcggcggtcgcctgcgtcggcggcgggtccaacgccatcggtctcttccacgccttcatcccggacgcggacgtacgtctcatcggctgcgagcccgccgggcacggcatcgagaccggcgagcacgcggccaccctgtccgcgggcgagcccggcatcctgcacggctcgcggtcgtacgtcctccaggacgaggagggccagatcaccgagccctactcga